European Patent Specification EP 3 739 062 B1, published August 16, 2023. Title: RED BLOOD CELL LYSIS SOLUTION. Applicant: Gen-Probe Incorporated Linnen, Jeff Chelliserry, Jijumon Gao, Kui. The sequence listing filed with the application follows.

SEQUENCE LISTING (5 sequences)

SEQ ID NO: 1 - DNA, 19 bp, Artificial Sequence
  Synthetic Oligonucleotide
acagggaggtagtgacaag

SEQ ID NO: 2 - DNA, 49 bp, Artificial Sequence
  Synthetic Oligonucleotide
  promoter (1)..(27)
aatttaatacgactcactatagggagactggaattaccgcggctgctgg

SEQ ID NO: 3 - RNA, 20 nt, Artificial Sequence
  Synthetic Oligonucleotide
  misc_feature (1)..(20): 2' O-Methyl
acccuucccagaguaucaau

SEQ ID NO: 4 - DNA, 54 bp, Artificial Sequence
  Synthetic Oligonucleotide
  misc_feature (1)..(21): 2' O-Methyl
ggauuggguaauuugcgcgcctttaaaaaaaaaaaaaaaaaaaaaaaaaaaaaa

SEQ ID NO: 5 - RNA, 1205 nt, Artificial Sequence
  Synthetic Oligonucleotide
gggcgaauuggguaccgggcccccccucgaggucgacgcuuaguauaagcuuuuauacagcgaaacugcgaauggcucauuaaaacaguuauaguuuauuugauguucguuuuacauggauaaccgugguaauucuagggcuaauacaugcucgaggcgcguuuucgcguggcguuuauuagacuuuaaccaacccuucggguaaucggugauucauaauaaauuagcgaaucgcauggcuuugccggcgauguaucauucaaguuucugaccuaucagcuuuggacgguaggguauuggccaccggggcgacgacgggugacggggaauugggguucgauuccggagagggagccugagaaacggcuaccacaucuaaggaaggcagcaggcgcgcaaauuacccaauccugacacagggagguagugacaagaaauaacaauacagggcuuaaagucuuguaauuggaaugaugggaaucuaaacccuucccagaguaucaauuggagggcaagucuggugccagcagccgcgguaauuccagcuccaauagcguauauuaaaguuguugcaguuaagaagcucguaguugaauuucugccuugucauuaaucucgcuuccgagcguuuuuuuauugacuuggcaucuucuggauuuggugccuucggguacuauuuuccaggauuuacuuugagaaaacuagaguguuucaaacaggcauucgccuugaauacuacagcauggaauaaugaaguaggacuuugguucuauuuuguugguuauugagccagaguaaugguuaauaggagcaguugggggcauucguauuuaacugucagaggugaaauucuuagauuuguuaaagacgaacuacugcgaaagcauuugccaaggauguuuucauuaaucaagaacgaaaguuaggggaucgaagacgaucagauaccgucguaguccuaaccauaaacuaugccgacuagagauuggaggucgucaguuuaaacgacuccuucagcaccuugagagaaaucaaagucuuuggguucuggggggaguauggucgcaagucugaaacuuaaaggaauugacggaagggcaccaccaggcguggagccugcggcuuaauuugacucaacacgggaaaccucaccagguccagacauagagaggauugacagauugauagcucuuucuugaugaauu